European Patent Specification EP 4 012 029 B1, published May 29, 2024. Title: Method for capturing nucleic acid molecule, method for preparing nucleic acid library and sequencing method. Applicant: GeneMind Biosciences Company Limited. The sequence listing filed with the application follows.

SEQUENCE LISTING (4 sequences)

SEQ ID NO: 1 - DNA, 20 bp, Artificial Sequence
  Artificial Sequence
  misc_feature (1)..(20): Artificial sequence
agatgtgtataagagacagt

SEQ ID NO: 2 - DNA, 51 bp, Artificial Sequence
  Artificial Sequence
  misc_feature (1)..(51): Artificial Sequence
ctgtctcttatacacatctgagtggaactggatggtcgcaggtatcaagga

SEQ ID NO: 3 - DNA, 52 bp, Artificial Sequence
  Artificial Sequence
  misc_feature (1)..(52): Artificial Sequence
tccttgatacctgcgaccatccagttccactcagatgtgtataagagacagt

SEQ ID NO: 4 - DNA, 61 bp, Artificial Sequence
  Artificial Sequence
  misc_feature (1)..(61): Artificial Sequence
tttttttttttccttgatacctgcgaccatccagttccactcagatgtgtataagagacag